European Patent Application EP 4 631 957 A1, published October 15, 2025. Title: Peptide for cartilage regeneration and uses thereof. Applicant: CAREGEN CO., LTD. The sequence listing filed with the application follows.

SEQUENCE LISTING (13 sequences)

SEQ ID NO: 1 - protein, 6 aa, synthetic construct
TAVRVG

SEQ ID NO: 2 - DNA, 23 bp, synthetic construct
  source 1..23: mol_type = other DNA
ctatctggacgaagcagctggca

SEQ ID NO: 3 - DNA, 22 bp, synthetic construct
  source 1..22: mol_type = other DNA
atgggtgcaatgtcaatgatgg

SEQ ID NO: 4 - DNA, 20 bp, synthetic construct
  source 1..20: mol_type = other DNA
aactcagggcaggaggatgt

SEQ ID NO: 5 - DNA, 20 bp, synthetic construct
  source 1..20: mol_type = other DNA
tgtccttttggtcgtcgttc

SEQ ID NO: 6 - DNA, 20 bp, synthetic construct
  source 1..20: mol_type = other DNA
ccagcccgaacttgtaaaga

SEQ ID NO: 7 - DNA, 20 bp, synthetic construct
  source 1..20: mol_type = other DNA
tggacgcacaaccatcatac

SEQ ID NO: 8 - DNA, 20 bp, synthetic construct
  source 1..20: mol_type = other DNA
gcaggctatgagcagtgtga

SEQ ID NO: 9 - DNA, 20 bp, synthetic construct
  source 1..20: mol_type = other DNA
gcatacctcggaagcagaag

SEQ ID NO: 10 - DNA, 20 bp, synthetic construct
  source 1..20: mol_type = other DNA
accacagtccatgccatcac

SEQ ID NO: 11 - DNA, 20 bp, synthetic construct
  source 1..20: mol_type = other DNA
tccaccaccctgttgctgta

SEQ ID NO: 12 - DNA, 20 bp, synthetic construct
  source 1..20: mol_type = other DNA
gcggaggaagtcggtgaaga

SEQ ID NO: 13 - DNA, 20 bp, synthetic construct
  source 1..20: mol_type = other DNA
ccctctcgcttcaggtcagc